European Patent Specification EP 4 010 472 B1, published January 1, 2025. Title: METHOD AND APPARATUS FOR SINGLE-CELL ANALYSIS FOR DETERMINING A CELL TRAJECTORY. Applicant: MISSION BIO, INC. Application PCT/US2020/045001. The sequence listing filed with the application follows.

SEQUENCE LISTING (184 sequences)

SEQ ID NO: 1 - DNA, 35 bp, Artificial Sequence
  Description of Artificial Sequence: Synthetic primer
gtactcgcagtagtctggttgtcctcgtcctcctt

SEQ ID NO: 2 - DNA, 44 bp, Artificial Sequence
  Description of Artificial Sequence: Synthetic primer
gtactcgcagtagtccggtatcctcgaattcaaagtatcaaagt

SEQ ID NO: 3 - DNA, 34 bp, Artificial Sequence
  Description of Artificial Sequence: Synthetic primer
gtactcgcagtagtcggtggagtgccgcttctac

SEQ ID NO: 4 - DNA, 38 bp, Artificial Sequence
  Description of Artificial Sequence: Synthetic primer
gtactcgcagtagtcagccaatgactttgtggtgacat

SEQ ID NO: 5 - DNA, 37 bp, Artificial Sequence
  Description of Artificial Sequence: Synthetic primer
gtactcgcagtagtcgcgactttacccttcgactaga

SEQ ID NO: 6 - DNA, 35 bp, Artificial Sequence
  Description of Artificial Sequence: Synthetic primer
gtactcgcagtagtccggagtattgggaccaggag

SEQ ID NO: 7 - DNA, 35 bp, Artificial Sequence
  Description of Artificial Sequence: Synthetic primer
gtactcgcagtagtcctgaaagccagggagttggt

SEQ ID NO: 8 - DNA, 35 bp, Artificial Sequence
  Description of Artificial Sequence: Synthetic primer
gtactcgcagtagtcgaagtgtggccagaagtgga

SEQ ID NO: 9 - DNA, 34 bp, Artificial Sequence
  Description of Artificial Sequence: Synthetic primer
gtactcgcagtagtcggtgtccttgggtgctgat

SEQ ID NO: 10 - DNA, 34 bp, Artificial Sequence
  Description of Artificial Sequence: Synthetic primer
gtactcgcagtagtccgagtacgtgccacaccaa

SEQ ID NO: 11 - DNA, 38 bp, Artificial Sequence
  Description of Artificial Sequence: Synthetic primer
gtactcgcagtagtcggaagaggcatctcgtttgtact

SEQ ID NO: 12 - DNA, 37 bp, Artificial Sequence
  Description of Artificial Sequence: Synthetic primer
gtactcgcagtagtcgtggagaagctcattgctacga

SEQ ID NO: 13 - DNA, 43 bp, Artificial Sequence
  Description of Artificial Sequence: Synthetic primer
gtactcgcagtagtctttaaagatgaccagagcatccaaaaga

SEQ ID NO: 14 - DNA, 42 bp, Artificial Sequence
  Description of Artificial Sequence: Synthetic primer
gtactcgcagtagtccactatgggactgagtaacattctctt

SEQ ID NO: 15 - DNA, 38 bp, Artificial Sequence
  Description of Artificial Sequence: Synthetic primer
gtactcgcagtagtcctgctcagtgtgatccttgcata

SEQ ID NO: 16 - DNA, 37 bp, Artificial Sequence
  Description of Artificial Sequence: Synthetic primer
gtactcgcagtagtctccagaatcgaaggccatcaag

SEQ ID NO: 17 - DNA, 41 bp, Artificial Sequence
  Description of Artificial Sequence: Synthetic primer
gtactcgcagtagtccccaaccgatatcatttctgatctgt

SEQ ID NO: 18 - DNA, 35 bp, Artificial Sequence
  Description of Artificial Sequence: Synthetic primer
gtactcgcagtagtcccatgagcgacgtggctatt

SEQ ID NO: 19 - DNA, 34 bp, Artificial Sequence
  Description of Artificial Sequence: Synthetic primer
gtactcgcagtagtcgcagtcgggcattccttca

SEQ ID NO: 20 - DNA, 41 bp, Artificial Sequence
  Description of Artificial Sequence: Synthetic primer
gtactcgcagtagtcaattgtcatagtggacatctgcatca

SEQ ID NO: 21 - DNA, 36 bp, Artificial Sequence
  Description of Artificial Sequence: Synthetic primer
gtactcgcagtagtccaatcctgcatcccccatagt

SEQ ID NO: 22 - DNA, 35 bp, Artificial Sequence
  Description of Artificial Sequence: Synthetic primer
gtactcgcagtagtcggatgcgccaggaagtttca

SEQ ID NO: 23 - DNA, 36 bp, Artificial Sequence
  Description of Artificial Sequence: Synthetic primer
gtactcgcagtagtcgtaccgctgcatgatcagcta

SEQ ID NO: 24 - DNA, 35 bp, Artificial Sequence
  Description of Artificial Sequence: Synthetic primer
gtactcgcagtagtcccgtggagcaggtgaagaat

SEQ ID NO: 25 - DNA, 36 bp, Artificial Sequence
  Description of Artificial Sequence: Synthetic primer
gtactcgcagtagtcgcgagtatggagcagaaacga

SEQ ID NO: 26 - DNA, 34 bp, Artificial Sequence
  Description of Artificial Sequence: Synthetic primer
gtactcgcagtagtcgcacaagcagctgatccga

SEQ ID NO: 27 - DNA, 40 bp, Artificial Sequence
  Description of Artificial Sequence: Synthetic primer
gtactcgcagtagtccctcctccttacctagacaatgaga

SEQ ID NO: 28 - DNA, 33 bp, Artificial Sequence
  Description of Artificial Sequence: Synthetic primer
gtactcgcagtagtccatgtttgcgcagctggt

SEQ ID NO: 29 - DNA, 37 bp, Artificial Sequence
  Description of Artificial Sequence: Synthetic primer
gtactcgcagtagtcgcctgtgtctccttgtgatgtt

SEQ ID NO: 30 - DNA, 33 bp, Artificial Sequence
  Description of Artificial Sequence: Synthetic primer
gtactcgcagtagtcaggactgcctgccccata

SEQ ID NO: 31 - DNA, 38 bp, Artificial Sequence
  Description of Artificial Sequence: Synthetic primer
gtactcgcagtagtcccaattggaacctgggatcaagt

SEQ ID NO: 32 - DNA, 39 bp, Artificial Sequence
  Description of Artificial Sequence: Synthetic primer
gtactcgcagtagtcgaagatgtaccaggtggagttcaa

SEQ ID NO: 33 - DNA, 38 bp, Artificial Sequence
  Description of Artificial Sequence: Synthetic primer
gtactcgcagtagtcgaaccgaagacgtgtttgcaaat

SEQ ID NO: 34 - DNA, 35 bp, Artificial Sequence
  Description of Artificial Sequence: Synthetic primer
gtactcgcagtagtctcaagagcgtgccctacttc

SEQ ID NO: 35 - DNA, 36 bp, Artificial Sequence
  Description of Artificial Sequence: Synthetic primer
gtactcgcagtagtcggccagaagagctgagacatc

SEQ ID NO: 36 - DNA, 38 bp, Artificial Sequence
  Description of Artificial Sequence: Synthetic primer
gtactcgcagtagtccgtcgtgtctcaagatctagctt

SEQ ID NO: 37 - DNA, 38 bp, Artificial Sequence
  Description of Artificial Sequence: Synthetic primer
gtactcgcagtagtcgtggatgactgagtacctgaacc

SEQ ID NO: 38 - DNA, 39 bp, Artificial Sequence
  Description of Artificial Sequence: Synthetic primer
gtactcgcagtagtccgagctatagaagaatcaccagca

SEQ ID NO: 39 - DNA, 43 bp, Artificial Sequence
  Description of Artificial Sequence: Synthetic primer
gtactcgcagtagtcccaagtgtccatacctcaatttctttca

SEQ ID NO: 40 - DNA, 33 bp, Artificial Sequence
  Description of Artificial Sequence: Synthetic primer
gtactcgcagtagtcgccctgcacgtggtgtaa

SEQ ID NO: 41 - DNA, 38 bp, Artificial Sequence
  Description of Artificial Sequence: Synthetic primer
gtactcgcagtagtcagtacaggatgcttgccaaaaga

SEQ ID NO: 42 - DNA, 41 bp, Artificial Sequence
  Description of Artificial Sequence: Synthetic primer
gtactcgcagtagtctgccgagctaaattacacattgatga

SEQ ID NO: 43 - DNA, 42 bp, Artificial Sequence
  Description of Artificial Sequence: Synthetic primer
gtactcgcagtagtcctaaacatctgcctgatctcatagagt

SEQ ID NO: 44 - DNA, 38 bp, Artificial Sequence
  Description of Artificial Sequence: Synthetic primer
gtactcgcagtagtcgaggccagcagtaaaacaacatc

SEQ ID NO: 45 - DNA, 38 bp, Artificial Sequence
  Description of Artificial Sequence: Synthetic primer
gtactcgcagtagtcgagcagagatacacgtgccatat

SEQ ID NO: 46 - DNA, 41 bp, Artificial Sequence
  Description of Artificial Sequence: Synthetic primer
gtactcgcagtagtcggactaacatgttcaatgtgggacaa

SEQ ID NO: 47 - DNA, 35 bp, Artificial Sequence
  Description of Artificial Sequence: Synthetic primer
gtactcgcagtagtcggaagtggtgctggttagga

SEQ ID NO: 48 - DNA, 38 bp, Artificial Sequence
  Description of Artificial Sequence: Synthetic primer
gtactcgcagtagtcagcgtgcagataatgacaaggaa

SEQ ID NO: 49 - DNA, 35 bp, Artificial Sequence
  Description of Artificial Sequence: Synthetic primer
gtactcgcagtagtccgatgggctcagctttcaga

SEQ ID NO: 50 - DNA, 36 bp, Artificial Sequence
  Description of Artificial Sequence: Synthetic primer
gtactcgcagtagtccgtcatgaagggtccttccaa

SEQ ID NO: 51 - DNA, 35 bp, Artificial Sequence
  Description of Artificial Sequence: Synthetic primer
gtactcgcagtagtcgctgggcttcacggacatag

SEQ ID NO: 52 - DNA, 37 bp, Artificial Sequence
  Description of Artificial Sequence: Synthetic primer
gtactcgcagtagtcagagtttgtatgccgcaagaca

SEQ ID NO: 53 - DNA, 41 bp, Artificial Sequence
  Description of Artificial Sequence: Synthetic primer
gtactcgcagtagtcgtgaacagaaaacttggaacgaaagt

SEQ ID NO: 54 - DNA, 35 bp, Artificial Sequence
  Description of Artificial Sequence: Synthetic primer
gtactcgcagtagtcggactttgaggcgggtgttt

SEQ ID NO: 55 - DNA, 41 bp, Artificial Sequence
  Description of Artificial Sequence: Synthetic primer
gtactcgcagtagtcagtacctccagaacagatttgagagt

SEQ ID NO: 56 - DNA, 35 bp, Artificial Sequence
  Description of Artificial Sequence: Synthetic primer
gtactcgcagtagtcggaggaatgtcagcaccaga

SEQ ID NO: 57 - DNA, 38 bp, Artificial Sequence
  Description of Artificial Sequence: Synthetic primer
gtactcgcagtagtcccagagcaggcagatgaaatacc

SEQ ID NO: 58 - DNA, 36 bp, Artificial Sequence
  Description of Artificial Sequence: Synthetic primer
gtactcgcagtagtcgtgtgcttgtggactctcaca

SEQ ID NO: 59 - DNA, 58 bp, Artificial Sequence
  Description of Artificial Sequence: Synthetic primer
gtctcgtgggctcggagatgtgtataagagacagagtctgaggtccagtagaagtgtt

SEQ ID NO: 60 - DNA, 62 bp, Artificial Sequence
  Description of Artificial Sequence: Synthetic primer
gtctcgtgggctcggagatgtgtataagagacaggagatgagataaaacccatcacagttga

SEQ ID NO: 61 - DNA, 55 bp, Artificial Sequence
  Description of Artificial Sequence: Synthetic primer
gtctcgtgggctcggagatgtgtataagagacaggggtgccgtagttggagataa

SEQ ID NO: 62 - DNA, 54 bp, Artificial Sequence
  Description of Artificial Sequence: Synthetic primer
gtctcgtgggctcggagatgtgtataagagacagtgcaggagtgtcagctttgt

SEQ ID NO: 63 - DNA, 54 bp, Artificial Sequence
  Description of Artificial Sequence: Synthetic primer
gtctcgtgggctcggagatgtgtataagagacaggggatccaggtgacccaaag

SEQ ID NO: 64 - DNA, 55 bp, Artificial Sequence
  Description of Artificial Sequence: Synthetic primer
gtctcgtgggctcggagatgtgtataagagacagccacgtcgcagccatacatta

SEQ ID NO: 65 - DNA, 58 bp, Artificial Sequence
  Description of Artificial Sequence: Synthetic primer
gtctcgtgggctcggagatgtgtataagagacagcttgtttcactctcacacccagat

SEQ ID NO: 66 - DNA, 62 bp, Artificial Sequence
  Description of Artificial Sequence: Synthetic primer
gtctcgtgggctcggagatgtgtataagagacagtcgtttggctggatcatagattaacatt

SEQ ID NO: 67 - DNA, 58 bp, Artificial Sequence
  Description of Artificial Sequence: Synthetic primer
gtctcgtgggctcggagatgtgtataagagacagaatagccctggtaggtaactctgt

SEQ ID NO: 68 - DNA, 59 bp, Artificial Sequence
  Description of Artificial Sequence: Synthetic primer
gtctcgtgggctcggagatgtgtataagagacagcattgaattcttcctggatgccaaa

SEQ ID NO: 69 - DNA, 59 bp, Artificial Sequence
  Description of Artificial Sequence: Synthetic primer
gtctcgtgggctcggagatgtgtataagagacaggcctccattaaatctcgaccatagg

SEQ ID NO: 70 - DNA, 54 bp, Artificial Sequence
  Description of Artificial Sequence: Synthetic primer
gtctcgtgggctcggagatgtgtataagagacaggtatgtgccctgctccttcc

SEQ ID NO: 71 - DNA, 56 bp, Artificial Sequence
  Description of Artificial Sequence: Synthetic primer
gtctcgtgggctcggagatgtgtataagagacagtgctttgcgttggacattcaag

SEQ ID NO: 72 - DNA, 55 bp, Artificial Sequence
  Description of Artificial Sequence: Synthetic primer
gtctcgtgggctcggagatgtgtataagagacagctagctcactcaggctttggt

SEQ ID NO: 73 - DNA, 53 bp, Artificial Sequence
  Description of Artificial Sequence: Synthetic primer
gtctcgtgggctcggagatgtgtataagagacagcattgcgacaggcacactc

SEQ ID NO: 74 - DNA, 56 bp, Artificial Sequence
  Description of Artificial Sequence: Synthetic primer
gtctcgtgggctcggagatgtgtataagagacagtgtagggaagtgatgggagagg

SEQ ID NO: 75 - DNA, 55 bp, Artificial Sequence
  Description of Artificial Sequence: Synthetic primer
gtctcgtgggctcggagatgtgtataagagacagttgggccagttttccttgtct

SEQ ID NO: 76 - DNA, 54 bp, Artificial Sequence
  Description of Artificial Sequence: Synthetic primer
gtctcgtgggctcggagatgtgtataagagacagctcacgttggtccacatcct

SEQ ID NO: 77 - DNA, 56 bp, Artificial Sequence
  Description of Artificial Sequence: Synthetic primer
gtctcgtgggctcggagatgtgtataagagacaggtgtagtcagacgagcactcat

SEQ ID NO: 78 - DNA, 54 bp, Artificial Sequence
  Description of Artificial Sequence: Synthetic primer
gtctcgtgggctcggagatgtgtataagagacaggtggtggcctctccttgttt

SEQ ID NO: 79 - DNA, 60 bp, Artificial Sequence
  Description of Artificial Sequence: Synthetic primer
gtctcgtgggctcggagatgtgtataagagacagtgtctctctttcctcttctgttccta

SEQ ID NO: 80 - DNA, 52 bp, Artificial Sequence
  Description of Artificial Sequence: Synthetic primer
gtctcgtgggctcggagatgtgtataagagacagctctggctctccgtcgtt

SEQ ID NO: 81 - DNA, 53 bp, Artificial Sequence
  Description of Artificial Sequence: Synthetic primer
gtctcgtgggctcggagatgtgtataagagacaggtagccctcagcctgacat

SEQ ID NO: 82 - DNA, 57 bp, Artificial Sequence
  Description of Artificial Sequence: Synthetic primer
gtctcgtgggctcggagatgtgtataagagacagtctatagagtcgccaccctgatg

SEQ ID NO: 83 - DNA, 58 bp, Artificial Sequence
  Description of Artificial Sequence: Synthetic primer
gtctcgtgggctcggagatgtgtataagagacagaattccaaatgagctctccaacca

SEQ ID NO: 84 - DNA, 60 bp, Artificial Sequence
  Description of Artificial Sequence: Synthetic primer
gtctcgtgggctcggagatgtgtataagagacagctctctcatgatcgtctttagccttt

SEQ ID NO: 85 - DNA, 56 bp, Artificial Sequence
  Description of Artificial Sequence: Synthetic primer
gtctcgtgggctcggagatgtgtataagagacagcaagctatagcaagccaggact

SEQ ID NO: 86 - DNA, 57 bp, Artificial Sequence
  Description of Artificial Sequence: Synthetic primer
gtctcgtgggctcggagatgtgtataagagacaggctccttcgtgtcctctttgtag

SEQ ID NO: 87 - DNA, 58 bp, Artificial Sequence
  Description of Artificial Sequence: Synthetic primer
gtctcgtgggctcggagatgtgtataagagacaggcttctccaaagatgatgctgtgt

SEQ ID NO: 88 - DNA, 56 bp, Artificial Sequence
  Description of Artificial Sequence: Synthetic primer
gtctcgtgggctcggagatgtgtataagagacagacattcctcgatgtccccttct

SEQ ID NO: 89 - DNA, 56 bp, Artificial Sequence
  Description of Artificial Sequence: Synthetic primer
gtctcgtgggctcggagatgtgtataagagacagccatgtgatctgacaccctgaa

SEQ ID NO: 90 - DNA, 57 bp, Artificial Sequence
  Description of Artificial Sequence: Synthetic primer
gtctcgtgggctcggagatgtgtataagagacaggatttttgtggcacagtctcact

SEQ ID NO: 91 - DNA, 55 bp, Artificial Sequence
  Description of Artificial Sequence: Synthetic primer
gtctcgtgggctcggagatgtgtataagagacagggaaggacttgctccctcaaa

SEQ ID NO: 92 - DNA, 59 bp, Artificial Sequence
  Description of Artificial Sequence: Synthetic primer
gtctcgtgggctcggagatgtgtataagagacaggattgagcatccaccaagaactttt

SEQ ID NO: 93 - DNA, 53 bp, Artificial Sequence
  Description of Artificial Sequence: Synthetic primer
gtctcgtgggctcggagatgtgtataagagacagggctgcgatttgcttcaca

SEQ ID NO: 94 - DNA, 56 bp, Artificial Sequence
  Description of Artificial Sequence: Synthetic primer
gtctcgtgggctcggagatgtgtataagagacagtgagtcatctgcggtactgtct

SEQ ID NO: 95 - DNA, 55 bp, Artificial Sequence
  Description of Artificial Sequence: Synthetic primer
gtctcgtgggctcggagatgtgtataagagacagggccaaactgagcagagtctt

SEQ ID NO: 96 - DNA, 56 bp, Artificial Sequence
  Description of Artificial Sequence: Synthetic primer
gtctcgtgggctcggagatgtgtataagagacagtcttcggagtttgggtttgctt

SEQ ID NO: 97 - DNA, 55 bp, Artificial Sequence
  Description of Artificial Sequence: Synthetic primer
gtctcgtgggctcggagatgtgtataagagacagttgtgccagctcttcaacaga

SEQ ID NO: 98 - DNA, 56 bp, Artificial Sequence
  Description of Artificial Sequence: Synthetic primer
gtctcgtgggctcggagatgtgtataagagacagcaactccaggcttgtagctgtc

SEQ ID NO: 99 - DNA, 58 bp, Artificial Sequence
  Description of Artificial Sequence: Synthetic primer
gtctcgtgggctcggagatgtgtataagagacagggagaaaatcaagtcgtgctgaat

SEQ ID NO: 100 - DNA, 54 bp, Artificial Sequence
  Description of Artificial Sequence: Synthetic primer
gtctcgtgggctcggagatgtgtataagagacagcatggtcacagagccacctt

SEQ ID NO: 101 - DNA, 56 bp, Artificial Sequence
  Description of Artificial Sequence: Synthetic primer
gtctcgtgggctcggagatgtgtataagagacagcccacacatatgccatggtgat

SEQ ID NO: 102 - DNA, 61 bp, Artificial Sequence
  Description of Artificial Sequence: Synthetic primer
gtctcgtgggctcggagatgtgtataagagacagacagaaggtgacttgggcatagatata

SEQ ID NO: 103 - DNA, 54 bp, Artificial Sequence
  Description of Artificial Sequence: Synthetic primer
gtctcgtgggctcggagatgtgtataagagacagagctccaaggacagctagga

SEQ ID NO: 104 - DNA, 55 bp, Artificial Sequence
  Description of Artificial Sequence: Synthetic primer
gtctcgtgggctcggagatgtgtataagagacaggagtggatttcccgtgtagca

SEQ ID NO: 105 - DNA, 58 bp, Artificial Sequence
  Description of Artificial Sequence: Synthetic primer
gtctcgtgggctcggagatgtgtataagagacagcttagggagtgggagaagtcaaag

SEQ ID NO: 106 - DNA, 56 bp, Artificial Sequence
  Description of Artificial Sequence: Synthetic primer
gtctcgtgggctcggagatgtgtataagagacaggatttgacggctcctctactgt

SEQ ID NO: 107 - DNA, 55 bp, Artificial Sequence
  Description of Artificial Sequence: Synthetic primer
gtctcgtgggctcggagatgtgtataagagacagacaaaacctcgtccacggaat

SEQ ID NO: 108 - DNA, 55 bp, Artificial Sequence
  Description of Artificial Sequence: Synthetic primer
gtctcgtgggctcggagatgtgtataagagacagatggctgtctgatggcattga

SEQ ID NO: 109 - DNA, 57 bp, Artificial Sequence
  Description of Artificial Sequence: Synthetic primer
gtctcgtgggctcggagatgtgtataagagacagttttcccaatgtagccagtgtca

SEQ ID NO: 110 - DNA, 56 bp, Artificial Sequence
  Description of Artificial Sequence: Synthetic primer
gtctcgtgggctcggagatgtgtataagagacagggcgagttggattttggactga

SEQ ID NO: 111 - DNA, 54 bp, Artificial Sequence
  Description of Artificial Sequence: Synthetic primer
gtctcgtgggctcggagatgtgtataagagacagcggtgtgctcctcactgtaa

SEQ ID NO: 112 - DNA, 62 bp, Artificial Sequence
  Description of Artificial Sequence: Synthetic primer
gtctcgtgggctcggagatgtgtataagagacagtcaatagcttgttgaactgcatgatgta

SEQ ID NO: 113 - DNA, 53 bp, Artificial Sequence
  Description of Artificial Sequence: Synthetic primer
gtctcgtgggctcggagatgtgtataagagacagtcagcaggctggcatttgt

SEQ ID NO: 114 - DNA, 59 bp, Artificial Sequence
  Description of Artificial Sequence: Synthetic primer
gtctcgtgggctcggagatgtgtataagagacagtcacacatatgattaggccaactgt

SEQ ID NO: 115 - DNA, 54 bp, Artificial Sequence
  Description of Artificial Sequence: Synthetic primer
gtctcgtgggctcggagatgtgtataagagacagagctccacagcatcgatgtc

SEQ ID NO: 116 - DNA, 56 bp, Artificial Sequence
  Description of Artificial Sequence: Synthetic primer
gtctcgtgggctcggagatgtgtataagagacaggccagcgagatgagaaatagca

SEQ ID NO: 117 - DNA, 59 bp, Artificial Sequence
  Description of Artificial Sequence: Synthetic primer
gtctcgtgggctcggagatgtgtataagagacagatggaacttgctaaggaagaaaagt

SEQ ID NO: 118 - DNA, 55 bp, Artificial Sequence
  Description of Artificial Sequence: Synthetic primer
gtctcgtgggctcggagatgtgtataagagacaggttttgtttcctggagggacc

SEQ ID NO: 119 - DNA, 55 bp, Artificial Sequence
  Description of Artificial Sequence: Synthetic primer
gtctcgtgggctcggagatgtgtataagagacagcgggaatgggagacaaagtca

SEQ ID NO: 120 - DNA, 59 bp, Artificial Sequence
  Description of Artificial Sequence: Synthetic primer
gtctcgtgggctcggagatgtgtataagagacagatttcagtgtccttgtctgttcttc

SEQ ID NO: 121 - DNA, 55 bp, Artificial Sequence
  Description of Artificial Sequence: Synthetic primer
gtctcgtgggctcggagatgtgtataagagacagtactctcctcttttgcacccc

SEQ ID NO: 122 - DNA, 62 bp, Artificial Sequence
  Description of Artificial Sequence: Synthetic primer
gtctcgtgggctcggagatgtgtataagagacagttttgggagaattaagtttgatagatgc

SEQ ID NO: 123 - DNA, 56 bp, Artificial Sequence
  Description of Artificial Sequence: Synthetic primer
gtctcgtgggctcggagatgtgtataagagacaggcagatgccttcttcgttatga

SEQ ID NO: 124 - DNA, 56 bp, Artificial Sequence
  Description of Artificial Sequence: Synthetic primer
gtctcgtgggctcggagatgtgtataagagacagatatgcaaagcagaaaccctcg

SEQ ID NO: 125 - DNA, 55 bp, Artificial Sequence
  Description of Artificial Sequence: Synthetic primer
gtctcgtgggctcggagatgtgtataagagacagctcagcatccaacaaggcact

SEQ ID NO: 126 - DNA, 55 bp, Artificial Sequence
  Description of Artificial Sequence: Synthetic primer
gtctcgtgggctcggagatgtgtataagagacagtggactccaagatggcaagct

SEQ ID NO: 127 - DNA, 54 bp, Artificial Sequence
  Description of Artificial Sequence: Synthetic primer
gtctcgtgggctcggagatgtgtataagagacagggctggccaaacataagcag

SEQ ID NO: 128 - DNA, 60 bp, Artificial Sequence
  Description of Artificial Sequence: Synthetic primer
gtctcgtgggctcggagatgtgtataagagacagatgcctttgataatgatttgatgcac

SEQ ID NO: 129 - DNA, 59 bp, Artificial Sequence
  Description of Artificial Sequence: Synthetic primer
gtctcgtgggctcggagatgtgtataagagacaggtgtctcaagatctagcttctcttc

SEQ ID NO: 130 - DNA, 56 bp, Artificial Sequence
  Description of Artificial Sequence: Synthetic primer
gtctcgtgggctcggagatgtgtataagagacagctcaggttcagggaggaaaagt

SEQ ID NO: 131 - DNA, 56 bp, Artificial Sequence
  Description of Artificial Sequence: Synthetic primer
gtctcgtgggctcggagatgtgtataagagacagcagccatttgtgttgttgtgtg

SEQ ID NO: 132 - DNA, 54 bp, Artificial Sequence
  Description of Artificial Sequence: Synthetic primer
gtctcgtgggctcggagatgtgtataagagacagagtggttcagcccgagaact

SEQ ID NO: 133 - DNA, 62 bp, Artificial Sequence
  Description of Artificial Sequence: Synthetic primer
gtctcgtgggctcggagatgtgtataagagacagaaaacccaagcttagatttattgaaagg

SEQ ID NO: 134 - DNA, 60 bp, Artificial Sequence
  Description of Artificial Sequence: Synthetic primer
gtctcgtgggctcggagatgtgtataagagacagatatgttcctaaaacatccctgagtt

SEQ ID NO: 135 - DNA, 54 bp, Artificial Sequence
  Description of Artificial Sequence: Synthetic primer
gtctcgtgggctcggagatgtgtataagagacagtgccaagctgtccccttctc

SEQ ID NO: 136 - DNA, 59 bp, Artificial Sequence
  Description of Artificial Sequence: Synthetic primer
gtctcgtgggctcggagatgtgtataagagacagttaatgcctcagaactttggtgtca

SEQ ID NO: 137 - DNA, 60 bp, Artificial Sequence
  Description of Artificial Sequence: Synthetic primer
gtctcgtgggctcggagatgtgtataagagacagttttaaggttatgtgatttctcccca

SEQ ID NO: 138 - DNA, 54 bp, Artificial Sequence
  Description of Artificial Sequence: Synthetic primer
gtctcgtgggctcggagatgtgtataagagacagctgcgtcacaccattgctat

SEQ ID NO: 139 - DNA, 58 bp, Artificial Sequence
  Description of Artificial Sequence: Synthetic primer
gtctcgtgggctcggagatgtgtataagagacagccattttccttgtcctagaacctt

SEQ ID NO: 140 - DNA, 59 bp, Artificial Sequence
  Description of Artificial Sequence: Synthetic primer
gtctcgtgggctcggagatgtgtataagagacagcattgtctgtagctatgattagggc

SEQ ID NO: 141 - DNA, 55 bp, Artificial Sequence
  Description of Artificial Sequence: Synthetic primer
gtctcgtgggctcggagatgtgtataagagacagtgggaagatgccagaagtgga

SEQ ID NO: 142 - DNA, 54 bp, Artificial Sequence
  Description of Artificial Sequence: Synthetic primer
gtctcgtgggctcggagatgtgtataagagacagcacagagttgatgagacgcg

SEQ ID NO: 143 - DNA, 54 bp, Artificial Sequence
  Description of Artificial Sequence: Synthetic primer
gtctcgtgggctcggagatgtgtataagagacagttccgaaagagctggtccca

SEQ ID NO: 144 - DNA, 54 bp, Artificial Sequence
  Description of Artificial Sequence: Synthetic primer
gtctcgtgggctcggagatgtgtataagagacagcgtagctggcgatgttgaaa

SEQ ID NO: 145 - DNA, 56 bp, Artificial Sequence
  Description of Artificial Sequence: Synthetic primer
gtctcgtgggctcggagatgtgtataagagacagcagcctccaactggtatcttca

SEQ ID NO: 146 - DNA, 56 bp, Artificial Sequence
  Description of Artificial Sequence: Synthetic primer
gtctcgtgggctcggagatgtgtataagagacagcttcgaaaagcagtctgtagca

SEQ ID NO: 147 - DNA, 56 bp, Artificial Sequence
  Description of Artificial Sequence: Synthetic primer
gtctcgtgggctcggagatgtgtataagagacagcctttcccactgtcctcatctg

SEQ ID NO: 148 - DNA, 53 bp, Artificial Sequence
  Description of Artificial Sequence: Synthetic primer
gtctcgtgggctcggagatgtgtataagagacagagccctgtgctcgggaagt

SEQ ID NO: 149 - DNA, 66 bp, Artificial Sequence
  Description of Artificial Sequence: Synthetic primer
gtctcgtgggctcggagatgtgtataagagacagaactagatttagaatagaaatgaacaaagcag

SEQ ID NO: 150 - DNA, 54 bp, Artificial Sequence
  Description of Artificial Sequence: Synthetic primer
gtctcgtgggctcggagatgtgtataagagacagcgtgcatcatggcaaagtga

SEQ ID NO: 151 - DNA, 42 bp, Artificial Sequence
  Description of Artificial Sequence: Synthetic primer
gtactcgcagtagtcgaccccatctgttaaattttatagggc

SEQ ID NO: 152 - DNA, 43 bp, Artificial Sequence
  Description of Artificial Sequence: Synthetic primer
gtactcgcagtagtccctggccttatgatgttttaaagaaaag

SEQ ID NO: 153 - DNA, 35 bp, Artificial Sequence
  Description of Artificial Sequence: Synthetic primer
gtactcgcagtagtctgaggtggactatcgccaga

SEQ ID NO: 154 - DNA, 37 bp, Artificial Sequence
  Description of Artificial Sequence: Synthetic primer
gtactcgcagtagtccagtgtacttcagttggtgcac

SEQ ID NO: 155 - DNA, 36 bp, Artificial Sequence
  Description of Artificial Sequence: Synthetic primer
gtactcgcagtagtctacctcttcctcccactccag

SEQ ID NO: 156 - DNA, 39 bp, Artificial Sequence
  Description of Artificial Sequence: Synthetic primer
gtactcgcagtagtctctcttattgactgttgtgcatgc

SEQ ID NO: 157 - DNA, 38 bp, Artificial Sequence
  Description of Artificial Sequence: Synthetic primer
gtactcgcagtagtcgctgaagtactgaagccatgaca

SEQ ID NO: 158 - DNA, 36 bp, Artificial Sequence
  Description of Artificial Sequence: Synthetic primer
gtactcgcagtagtccatagtcgctgcttgatcgct

SEQ ID NO: 159 - DNA, 37 bp, Artificial Sequence
  Description of Artificial Sequence: Synthetic primer
gtactcgcagtagtcgctccgtaaatgctacgaagtg

SEQ ID NO: 160 - DNA, 43 bp, Artificial Sequence
  Description of Artificial Sequence: Synthetic primer
gtactcgcagtagtctcttctaatttccaagaaaatctttggc

SEQ ID NO: 161 - DNA, 38 bp, Artificial Sequence
  Description of Artificial Sequence: Synthetic primer
gtactcgcagtagtcacctgtctgcaaatgctctgttg

SEQ ID NO: 162 - DNA, 35 bp, Artificial Sequence
  Description of Artificial Sequence: Synthetic primer
gtactcgcagtagtcaagaggcgcaggtggaacat

SEQ ID NO: 163 - DNA, 35 bp, Artificial Sequence
  Description of Artificial Sequence: Synthetic primer
gtactcgcagtagtctttctgccattacgtccagc

SEQ ID NO: 164 - DNA, 38 bp, Artificial Sequence
  Description of Artificial Sequence: Synthetic primer
gtactcgcagtagtcaatggaagagaactttgccgttg

SEQ ID NO: 165 - DNA, 36 bp, Artificial Sequence
  Description of Artificial Sequence: Synthetic primer
gtactcgcagtagtctctactgtacaccccatccca

SEQ ID NO: 166 - DNA, 36 bp, Artificial Sequence
  Description of Artificial Sequence: Synthetic primer
gtactcgcagtagtcgccactcatggtgttgatgct

SEQ ID NO: 167 - DNA, 36 bp, Artificial Sequence
  Description of Artificial Sequence: Synthetic primer
gtactcgcagtagtcggtccatagagcggttgattg

SEQ ID NO: 168 - DNA, 38 bp, Artificial Sequence
  Description of Artificial Sequence: Synthetic primer
gtactcgcagtagtccgcaaggtctagttcatttccaa

SEQ ID NO: 169 - DNA, 35 bp, Artificial Sequence
  Description of Artificial Sequence: Synthetic primer
gtactcgcagtagtcttgtgctaaacgctgggagg

SEQ ID NO: 170 - DNA, 36 bp, Artificial Sequence
  Description of Artificial Sequence: Synthetic primer
gtactcgcagtagtcctgctgcaccttgagtcagag

SEQ ID NO: 171 - DNA, 38 bp, Artificial Sequence
  Description of Artificial Sequence: Synthetic primer
gtactcgcagtagtcacaagttgttcagaagaagcctg

SEQ ID NO: 172 - DNA, 36 bp, Artificial Sequence
  Description of Artificial Sequence: Synthetic primer
gtactcgcagtagtcgcagagaagagtgtcgcaaaa

SEQ ID NO: 173 - DNA, 38 bp, Artificial Sequence
  Description of Artificial Sequence: Synthetic primer
gtactcgcagtagtctcccaaatccgagaaatggaaac

SEQ ID NO: 174 - DNA, 36 bp, Artificial Sequence
  Description of Artificial Sequence: Synthetic primer
gtactcgcagtagtcggccaggaaatcacatcctac

SEQ ID NO: 175 - DNA, 36 bp, Artificial Sequence
  Description of Artificial Sequence: Synthetic primer
gtactcgcagtagtccagcggaatgaccttctcctc

SEQ ID NO: 176 - DNA, 35 bp, Artificial Sequence
  Description of Artificial Sequence: Synthetic primer
gtactcgcagtagtctcgtcgatgcctatgacagc

SEQ ID NO: 177 - DNA, 40 bp, Artificial Sequence
  Description of Artificial Sequence: Synthetic primer
gtactcgcagtagtcttacctatacatctcagcatggccg

SEQ ID NO: 178 - DNA, 38 bp, Artificial Sequence
  Description of Artificial Sequence: Synthetic primer
gtactcgcagtagtcgaccaactgcaaagagtgattga

SEQ ID NO: 179 - DNA, 38 bp, Artificial Sequence
  Description of Artificial Sequence: Synthetic primer
gtactcgcagtagtcctggtgtaagaactcaggtctgt

SEQ ID NO: 180 - DNA, 38 bp, Artificial Sequence
  Description of Artificial Sequence: Synthetic primer
gtactcgcagtagtcggatcctaaagaaggcatccaaa

SEQ ID NO: 181 - DNA, 38 bp, Artificial Sequence
  Description of Artificial Sequence: Synthetic primer
gtactcgcagtagtcaatcggaagcctaactacagcga

SEQ ID NO: 182 - DNA, 34 bp, Artificial Sequence
  Description of Artificial Sequence: Synthetic primer
gtactcgcagtagtcagcctctgacccacgtcga

SEQ ID NO: 183 - DNA, 41 bp, Artificial Sequence
  Description of Artificial Sequence: Synthetic primer
gtactcgcagtagtccgagcaccattatagctgttaaaccg

SEQ ID NO: 184 - DNA, 36 bp, Artificial Sequence
  Description of Artificial Sequence: Synthetic primer
gtactcgcagtagtctcatgaccattccgtaccagc